European Patent Application EP 4 389 769 A1, published June 26, 2024. Title: ANTI-PTK7 SINGLE-DOMAIN ANTIBODY AND APPLICATION THEREOF. Applicant: NANOMAB TECHNOLOGY LIMITED. The sequence listing filed with the application follows.

SEQUENCE LISTING (31 sequences)

SEQ ID NO: 1 - protein, 130 aa, Camelus bactrianus
QVQLQESGGGSVQAGGSLRLSCTASGFTFDDYDMVWYRQAPGNEYEWLSTVSRGGNLYYADSVKGRFTISRDNAKNTVYLNMSRVKPEDTAVYYCAADLRSVPSTYRARTCRGRYCRDYWGQGTQVTVSS

SEQ ID NO: 2 - protein, 127 aa, Camelus bactrianus
QVQLQESGGGSVQAGGSLRLSCAASGYIWSRYCMGWFRQAPGKAREGVARFNSDGNTRYVDSVKGRFTISRDNAKNTLYLQMNNLQPEDTARYYCAADPRFDCGYDAVFNPTHFPYWGRGTQVTVSS

SEQ ID NO: 3 - protein, 127 aa, Camelus bactrianus
QVQLQESGGGSVQAGGSLRLSCAASGYIWSRYCMGWFRQAPGKAREGVARFNSDGNTRYVDSVKGRFTISRDNAKNTLYLQMNNLQPEDTARYYCAADPRFDCGYDAVFNPTHFPYWGQGTQVTVSS

SEQ ID NO: 4 - protein, 124 aa, Camelus bactrianus
QVQLQESGGGLVQPGGSLTLACAASGFAFSSYAMRWVRQAPGKGLEGVSSISAGGDETYYADFAKGRFTISRDNAKNTLYLQLNSLKTEDTAMYYCAKGDRNSPRYSSWPITPVGQGTQVTVSS

SEQ ID NO: 5 - DNA, 390 bp, Camelus bactrianus
  source 1..390: mol_type = other DNA
caggtgcagctgcaggagtctgggggaggctcggtacaggctggagggtctctgagactctcctgtacagcctctggattcacttttgatgattatgacatggtctggtaccgccaggctccagggaatgagtacgagtggctctcaactgttagtcgtggtggtaatttatactatgcagactctgtgaagggccgattcaccatctcccgagacaacgccaagaacacggtgtatcttaatatgagcagagtgaaacctgaggacacggccgtctattactgcgcggcagaccttcgctcggttccctcgacgtatcgggcgagaacttgtcgcggtcgttactgccgcgactactggggccaggggacccaggtcaccgtctcctca

SEQ ID NO: 6 - DNA, 381 bp, Camelus bactrianus
  source 1..381: mol_type = other DNA
caggtgcagctgcaggagtctggaggaggctcggtgcaggctggagggtctctgagactctcctgtgcagcctctggatacatctggagtaggtactgcatgggctggttccgccaggctccagggaaggcgcgcgagggggtcgcgcgctttaatagtgatggtaacacaaggtacgtagactccgtgaagggccgattcaccatctcccgagacaacgccaagaacactctgtatctgcaaatgaacaacctgcaacctgaggacactgccaggtactactgtgcggcagatcctcgcttcgattgcggctatgacgccgtgtttaacccgacgcactttccttactggggccgggggacccaggtcaccgtctcctca

SEQ ID NO: 7 - DNA, 381 bp, Camelus bactrianus
  source 1..381: mol_type = other DNA
caggtgcagctgcaggagtctgggggaggctcggtgcaggctggagggtctctgagactctcctgtgcagcctctggatacatctggagtaggtactgcatgggctggttccgccaggctccagggaaggcgcgcgagggggtcgcgcgctttaatagtgatggtaacacaaggtacgtagactccgtgaagggccgattcaccatctcccgagacaacgccaagaacactctgtatctgcaaatgaacaacctgcaacctgaggacactgccaggtactactgtgcggcagatcctcgcttcgattgcggctatgacgccgtgtttaacccgacgcactttccttactggggccaggggacccaggtcaccgtctcctca

SEQ ID NO: 8 - DNA, 372 bp, Camelus bactrianus
  source 1..372: mol_type = other DNA
caggtgcagctgcaggagtctggaggaggcttggtgcagcctggggggtctctgacactcgcctgtgcagcctctggattcgccttcagtagctatgccatgcgctgggtccgccaggctccagggaagggactcgagggggtctcaagtattagtgctggtggtgatgaaacatactatgcagacttcgcgaagggccgattcaccatctccagagacaacgccaagaatacgctgtatttgcagctgaacagcctgaaaactgaggacacggccatgtattactgtgcaaagggggatcgtaactcccccagatacagtagttggcccatcacacccgtaggtcaggggacccaggtcaccgtctcctca

SEQ ID NO: 9 - protein, 10 aa, Camelus bactrianus
GFTFDDYDMV

SEQ ID NO: 10 - protein, 10 aa, Camelus bactrianus
GYIWSRYCMG

SEQ ID NO: 11 - protein, 10 aa, Camelus bactrianus
GFAFSSYAMR

SEQ ID NO: 12 - protein, 7 aa, Camelus bactrianus
TVSRGGN

SEQ ID NO: 13 - protein, 7 aa, Camelus bactrianus
RFNSDGN

SEQ ID NO: 14 - protein, 8 aa, Camelus bactrianus
SISAGGDE

SEQ ID NO: 15 - protein, 24 aa, Camelus bactrianus
AADLRSVPSTYRARTCRGRYCRDY

SEQ ID NO: 16 - protein, 21 aa, Camelus bactrianus
AADPRFDCGYDAVFNPTHFPY

SEQ ID NO: 17 - protein, 24 aa, Camelus bactrianus
YYCAADPRFDCGYDAVFNPTHFPY

SEQ ID NO: 18 - protein, 17 aa, Camelus bactrianus
AKGDRNSPRYSSWPITP

SEQ ID NO: 19 - protein, 25 aa, Camelus bactrianus
QVQLQESGGGSVQAGGSLRLSCTAS

SEQ ID NO: 20 - protein, 25 aa, Camelus bactrianus
QVQLQESGGGSVQAGGSLRLSCAAS

SEQ ID NO: 21 - protein, 25 aa, Camelus bactrianus
QVQLQESGGGLVQPGGSLTLACAAS

SEQ ID NO: 22 - protein, 14 aa, Camelus bactrianus
WYRQAPGNEYEWLS

SEQ ID NO: 23 - protein, 14 aa, Camelus bactrianus
WFRQAPGKAREGVA

SEQ ID NO: 24 - protein, 14 aa, Camelus bactrianus
WVRQAPGKGLEGVS

SEQ ID NO: 25 - protein, 39 aa, Camelus bactrianus
LYYADSVKGRFTISRDNAKNTVYLNMSRVKPEDTAVYYC

SEQ ID NO: 26 - protein, 39 aa, Camelus bactrianus
TRYVDSVKGRFTISRDNAKNTLYLQMNNLQPEDTARYYC

SEQ ID NO: 27 - protein, 36 aa, Camelus bactrianus
TRYVDSVKGRFTISRDNAKNTLYLQMNNLQPEDTAR

SEQ ID NO: 28 - protein, 39 aa, Camelus bactrianus
TYYADFAKGRFTISRDNAKNTLYLQLNSLKTEDTAMYYC

SEQ ID NO: 29 - protein, 11 aa, Camelus bactrianus
WGQGTQVTVSS

SEQ ID NO: 30 - protein, 11 aa, Camelus bactrianus
WGRGTQVTVSS

SEQ ID NO: 31 - protein, 11 aa, Camelus bactrianus
VGQGTQVTVSS